European Patent Specification EP 4 068 985 B1, published March 27, 2024. Title: Method for preparing galacto-oligosaccharides from lactulose. Applicant: FrieslandCampina Nederland B.V. The sequence listing filed with the application follows.

SEQUENCE LISTING (4 sequences)

SEQ ID NO: 1 - protein, 696 aa, Cryptococcus terrestris
MIPASALLAAVPLLAQQVSAGILRRQNAAGSDSAAPDSIADASTGVVSSIATEAVSSGATGLVASVAMSFASSMATPTATVTGLSSETGAPSNTPMASASGSVPTTTSAVGSGDFDWVQTDGLPTITTTLATTNQDAITPTATGPVGGQGTPAVNFTDYSSSSLEQFWNDWVGEVEEPPFAYVPEPPNPYPLPNAPPPIYPEYYTKRPKDILPDYKFPKDFLFGWATAAQQWEGAVKADGKGPSIWDWASRFPGFIADNTTSDVGDLGYYLYKEDLARIAALGANVYSFSMFWTRIFPFGKADSPVNQAGIDFYHDLIDYSWSLGIEPVVTLFHWDTPLALQLEYGGFASERIIDDYVNYAETVFKAYNGSVHKWVTFNEPVVFCSQMAAPVNTTLPPNLNSTIYPYTCSYHLVLAHAKTVKRFRELNIQGQIAFKSDNFVGIPWREGNQEDIDAVERHQAYQIGIFAEPIYNTGDWPDIVKNDLSPDILPRFTDDEIAMIKCTADFFPIDGYRDGYVQAVPGGVEACVANISNPLWPACNQVNFYDSTPAGWAIGTFGNWPTTPWLQNTWQFVRPFLADLAKRYPTEGGIYLSEFGFSEPFENDKTFIYQITQDSGRTAYFNSYLGEVLKGIVEDGIPIKGVFGWSMVDNFEWNSGLSTRFGVQYVDYNSPTRQRTFKRSALEMSEFWNAHRCSA

SEQ ID NO: 2 - protein, 566 aa, Cryptococcus terrestris
ATTNQDAITPTATGPVGGQGTPAVNFTDYSSSSLEQFWNDWVGEVEEPPFAYVPEPPNPYPLPNAPPPIYPEYYTKRPKDILPDYKFPKDFLFGWATAAQQWEGAVKADGKGPSIWDWASRFPGFIADNTTSDVGDLGYYLYKEDLARIAALGANVYSFSMFWTRIFPFGKADSPVNQAGIDFYHDLIDYSWSLGIEPVVTLFHWDTPLALQLEYGGFASERIIDDYVNYAETVFKAYNGSVHKWVTFNEPVVFCSQMAAPVNTTLPPNLNSTIYPYTCSYHLVLAHAKTVKRFRELNIQGQIAFKSDNFVGIPWREGNQEDIDAVERHQAYQIGIFAEPIYNTGDWPDIVKNDLSPDILPRFTDDEIAMIKCTADFFPIDGYRDGYVQAVPGGVEACVANISNPLWPACNQVNFYDSTPAGWAIGTFGNWPTTPWLQNTWQFVRPFLADLAKRYPTEGGIYLSEFGFSEPFENDKTFIYQITQDSGRTAYFNSYLGEVLKGIVEDGIPIKGVFGWSMVDNFEWNSGLSTRFGVQYVDYNSPTRQRTFKRSALEMSEFWNAHRCSA

SEQ ID NO: 3 - protein, 560 aa, Cryptococcus terrestris
AITPTATGPVGGQGTPAVNFTDYSSSSLEQFWNDWVGEVEEPPFAYVPEPPNPYPLPNAPPPIYPEYYTKRPKDILPDYKFPKDFLFGWATAAQQWEGAVKADGKGPSIWDWASRFPGFIADNTTSDVGDLGYYLYKEDLARIAALGANVYSFSMFWTRIFPFGKADSPVNQAGIDFYHDLIDYSWSLGIEPVVTLFHWDTPLALQLEYGGFASERIIDDYVNYAETVFKAYNGSVHKWVTFNEPVVFCSQMAAPVNTTLPPNLNSTIYPYTCSYHLVLAHAKTVKRFRELNIQGQIAFKSDNFVGIPWREGNQEDIDAVERHQAYQIGIFAEPIYNTGDWPDIVKNDLSPDILPRFTDDEIAMIKCTADFFPIDGYRDGYVQAVPGGVEACVANISNPLWPACNQVNFYDSTPAGWAIGTFGNWPTTPWLQNTWQFVRPFLADLAKRYPTEGGIYLSEFGFSEPFENDKTFIYQITQDSGRTAYFNSYLGEVLKGIVEDGIPIKGVFGWSMVDNFEWNSGLSTRFGVQYVDYNSPTRQRTFKRSALEMSEFWNAHRCSA

SEQ ID NO: 4 - protein, 555 aa, Cryptococcus terrestris
ATGPVGGQGTPAVNFTDYSSSSLEQFWNDWVGEVEEPPFAYVPEPPNPYPLPNAPPPIYPEYYTKRPKDILPDYKFPKDFLFGWATAAQQWEGAVKADGKGPSIWDWASRFPGFIADNTTSDVGDLGYYLYKEDLARIAALGANVYSFSMFWTRIFPFGKADSPVNQAGIDFYHDLIDYSWSLGIEPVVTLFHWDTPLALQLEYGGFASERIIDDYVNYAETVFKAYNGSVHKWVTFNEPVVFCSQMAAPVNTTLPPNLNSTIYPYTCSYHLVLAHAKTVKRFRELNIQGQIAFKSDNFVGIPWREGNQEDIDAVERHQAYQIGIFAEPIYNTGDWPDIVKNDLSPDILPRFTDDEIAMIKCTADFFPIDGYRDGYVQAVPGGVEACVANISNPLWPACNQVNFYDSTPAGWAIGTFGNWPTTPWLQNTWQFVRPFLADLAKRYPTEGGIYLSEFGFSEPFENDKTFIYQITQDSGRTAYFNSYLGEVLKGIVEDGIPIKGVFGWSMVDNFEWNSGLSTRFGVQYVDYNSPTRQRTFKRSALEMSEFWNAHRCSA